European Patent Application EP 4 218 752 A1, published August 2, 2023. Title: 用于判断线粒体氧化磷酸化通路抑制剂抗癌效果的标志物. Applicant: 南京施江医药科技有限公司. The sequence listing filed with the application follows.

SEQUENCE LISTING (3 sequences)

SEQ ID NO: 1 - DNA, 2500 bp, Homo sapiens
tatccaagagctatcagcactcccatgtttattgtagcactgttcacaatagccaagatttggaagtactctaagtgtccattagcagatgaatggataaagacaatgtggtaatacacataatggagtactattcagtcataaagaagaattagatcctgtcatttgcaataacatggatggaactggaggtcataatgttgagtgaaataaaccaggcacagaaagacaaactttgcatgttctcacttatttatgggagctaaaaactaaaataactgaactcacagagatagagagtagaaggatggttacgagaggatgggaagggtagcgaggtgggtaggggggatgtggggatcattaatgggtataaaaaatagttagaggccaggcgcagtggctcacgcctgtaatcccagcactttgggaggccgaggtaggcggaacacctgaggagttcaagaccagcctggccaatatgatgaaaccccgtctctactaaaaatacaaaaattagctgggcgtgatggtgtgcacctgtagtcccagctgcttgggaggctgaggcaggagaatcgctggaacccaagaggtgaaggttgcagtgagctgagatcgcgtcactgcactccagcctgggtgacagagtgagactccacatcaaaaaaaaaaaaaaaaagttagaaagattgaataagacctaatatttgctagcacaacagggtgaatatagtaaaaaataatttatttgtaccttcaaaaataactagacaagtataattgggttgtttgtaacacacaaaaaataagtacttgaagtggtggataccccatttaccctgatgtgattattttgtattgcaggcctctatcagaatatctcatgtaacccataaatatatacacctactctgtacccacaaaaagtttttaaaaagaaaaataaatagcaaccgaaaaaaaaagagagggagaaaagaaaaaagaaaaaaaaatcaagtgcctggctgggtagaataaattctaaggccacaatgttactgaccatgggttttttggctctcagtgtatagaaattgacacaaggccaatagtcttcccaaacatgctttactggaacttacgccctggcataagggccacaacaaaagagagagcgaattctctggcttgctgactccttggaaaaaaccggtagggatttttttattaggcaaagcacaggaattgacgtcagaggcaggatgtgctgctgggcaaagcatacgagaagtggggtatgcaggtcagcattacttggttgcaatggttatcttgaggaatgggccaactggtggtctggccagtggcaacaaggctgtaaatcaattattcagcattccttcccaaggtgggacacccggcaacattgtttatctcctaaggccagttcctggaattaagtgaaaggatgactaatggacatgttgtcagtgaggtagtggtgtgggttttgtgaccagtgggaatgcacgaaagaatgctttagcggggagtgagctgaagccaagccccatccctactctgtctcaaagtgagttcagaaaaggggatttaaagaattctttttttttttttttttttttttgagacagagtcttgctctgtcgcccaggctggagtgcagtggcgccatcttggctcactgcaagctccgccccccgggttcatgccattctcctgcctcagcctcccaagtagctgggactgcaggtgcctaccaccaagcccagctaattttttgtattttttttttagtagagacggggtttcaccatgttagccaggatggtctcgatctcctgacctcgtgatctgcccgccttagcctcccaaagtgctgggattacaggcatgagcctccgcccccggccttaaataattcttaaaggaagtaaagttaactttgaaagaactatcaggatttggattgactgaaaggagtggggaagcttagggaggaggtgcttgccagacactgggtcatggcagtggtcggtgaagctgcagttgcctagggcagggatggagagagagtctgggcatgaggagagggtctcgggatgtttggctggactagattttacagaaagccttatccaggcttttaaaattactctttccagacttcatctgagactccttcttcagccaacattccttagccctgaatacatttcctatcctcatctttcccttcttttttttcctttcttttacatgtttaaatttaaaccattcttcgtgaccccttttcttgggagattcatggcaagaacgagaagaatgatggtgcttgttaggggatgtcctgtctctctgaactttggggtcctatgcattaaataattttcctgacgagctcaagtgctccctctggtctacaatccctggcggctggccttcatcccttgggcaagcattgcatacagctcatggccctccctctaccataccc

SEQ ID NO: 2 - DNA, 63 bp, Artificial Sequence
  sh-DNMT1#1
gatccggcccaatgagactgacatcaattcaagagattgatgtcagtctcattgggctttttg

SEQ ID NO: 3 - DNA, 64 bp, Artificial Sequence
  sh-DNMT1#2
gatccgggatgagtccatcaaggaagattcaagagatcttccttgatggactcatccttttttg